European Patent Specification EP 3 464 601 B1, published July 3, 2024. Title: TRANSGENIC PLANTS WITH INCREASED PHOTOSYNTHESIS EFFICIENCY AND GROWTH. Applicant: The Board of Trustees of the University of Illinois The Regents of the University of California. Application Not Yet Assigned. The sequence listing filed with the application follows.

SEQUENCE LISTING (68 sequences)

SEQ ID NO: 1 - DNA, 1059 bp, Arabidopsis thaliana
atcttttaatctcttcacttccacaacacaacacaaaacacatcactgatccttctctcatcctcagaaagaatggctcaaaccatgctgcttacttcaggcgtcaccgccggccattttttgaggaacaagagccctttggctcagcccaaagttcaccatctcttcctctctggaaactctccggttgcactaccatctaggagacaatcattcgttcctctcgctctcttcaaacccaaaaccaaagctgctcctaaaaaggttgagaagccgaagagcaaggttgaggatggcatctttggaacgtctggtgggattggtttcacaaaggcgaatgagctattcgttggtcgtgttgctatgatcggtttcgctgcatcgttgcttggtgaggcgttgacgggaaaagggatattagctcagctgaatctggagacagggataccgatttacgaagcagagccattgcttctcttcttcatcttgttcactctgttgggagccattggagctctcggagacagaggaaaattcgtcgacgatcctcccaccgggctcgagaaagccgtcattcctcccggcaaaaacgtccgatctgccctcggtctcaaagaacaaggtccattgtttgggttcacgaaggcgaacgagttattcgtaggaagattggcacagttgggaatagcattttcactgataggagagattattaccgggaaaggagcattagctcaactcaacattgagaccggtataccaattcaagatatcgaaccacttgtcctcttaaacgttgctttcttcttcttcgctgccattaatcctggtaatggaaaattcatcaccgatgatggtgaagaaagctaaattatcatgtacttaaatttagtagagagtgtgtgaccttctcttcatgttgagacaaaaggaaatggacagcttaaattgttgtaatacttatatccttttgtttttaacttggaattttctgattatatatagttttattacacctaagtgactaggtgattgatatcatctagcatctcttaacag

SEQ ID NO: 2 - DNA, 2385 bp, Arabidopsis thaliana
atttgcctccttcttcttcaaaccaatttcttcttcttcttctctcaggtttgagtctgaggcatcacaacagataaagtcttgaactttgatcaagaattctaaacggagtttttgctcttctcgtcggtgaaagaaaaatcgagatgggttcaactccgttttgctactctatcaatccatctccatcaaagcttgatttcacgaggacccatgtgtttagtcctgtttctaaacagttttacttagatttatcatcgttttccggaaaacccggaggagtatctgggtttaggagccgtcgagctttgctcggagtaaaggcggcgacggcgttagttgagaaggaggagaagagagaggcggtgacggagaagaagaagaaatcgagggttttagttgccggaggtggaatcggaggattggtgtttgctttagcggctaagaagaaaggattcgatgtgttagtgtttgagaaagatttgagtgctataagaggagaaggaaaatacagaggcccgattcaaatacagagcaacgctttagctgctttggaagctattgatattgaagttgctgaacaagttatggaagctgggtgtatcactggtgatcggattaacggtctcgttgatggtatctctggtacttggtatgtaaagtttgatactttcactcctgcggcgtcacggggacttcctgtgactagagtaattagtagaatgactctgcagcagattctagcacgtgcggttggagaagatgtgattagaaacgagagtaatgttgttgattttgaagattctggagataaggttactgtggtactcgagaatggtcaacgctatgaaggtgatctgcttgtgggtgcagatggcatttggtctaaggtgagaaataatttgtttggccgtagtgaagctacttattcaggctacacttgttacacggggattgcagattttataccagcggatatcgagtctgttggctaccgggttttcttgggacacaaacagtactttgtttcttcggatgttggtggtggaaaaatgcaatggtatgcatttcacgaggaaccagctggtggggctgatgctccaaatggtatgaagaaaaggttgtttgaaatatttgacggttggtgcgacaatgtactcgacttgttgcatgcgactgaggaggaagccattctgagaagagatatttatgatagaagtcctggttttacttggggtaaagggcgtgttacgctgctcggggattctatccatgcgatgcagccaaatatgggtcaaggtggatgcatggccattgaggatagttttcaactagcattggagcttgatgaagcatggaaacagagtgttgaaacgactacacctgttgatgttgtttcctctttgaaaagatatgaggaatctagaagactgagagtcgctattatccatgcaatggcgaggatggctgcaattatggcttccacttacaaagcatacttaggtgttgggcttggtcctctgtctttcttgacaaagtttagagtaccacatccaggaagagttggtggtagattcttcgttgacattgctatgccatcgatgcttgactgggtccttggaggtaacagtgaaaaactccaaggaaggccacctagttgcagactcactgacaaagccgatgaccggcttcgagagtggtttgaagatgacgatgctcttgaacgtactataaagggagaatggtatctaattccacacggcgacgattgttgcgtttcggaaacattatgtctaaccaaagatgaagatcaaccttgcatcgtcggaagcgaaccagatcaagattttcctggaatgcgcattgtgatcccttcgtctcaggtttcgaagatgcatgctcgtgtgatttacaaagacggagctttcttcttgatggatcttcgaagcgaacacggaacctatgtgaccgataacgaaggaagaagatatagagcaacaccgaattttcccgcgcggtttagatcgtccgacatcatcgagtttggttcagataagaaggcggcgtttagggtgaaagtaatcaggaaaactccgaaatcgacgaggaagaatgagagtaacaacgataaattacttcagacagcttgaaataagtaaaccgatggtgaaattaagtaattttaatcggtttggcagataatttgagtagtaattttctcaaaagaaaaaaaatctgctttcagctattccttgcatgacaatgtatatataggtctgaaacaaaatataaattatacaagacattaatcttcatttcttcaacttccaggcaacaataatctaattttgattactaaaaggtaattatattatcaaattgttt

SEQ ID NO: 3 - DNA, 1776 bp, Arabidopsis thaliana
gagatatttgggtggagaaaacaaccgcctaggacaaaaaaaaattgtgggtagaggaggaggaggaggctttgttcacacaccacacgacggaacattctcttccgagtcttatccaaagcaaaatcatattttgcttaaatatcttcttctccggctctgtctctgtctctcttcttcccgcggagctttcagtttttgtttggtattgcttggtgtggggaagattagatagtgtgaagaatggcagtagctacacattgtttcacttcaccttgtcatgaccgtattcgatttttctcaagtgatgatggtattggtaggcttggcattacaagaaagaggatcaatggcactttcttgctcaagattttacctccaatccaaagtgctgatctcagaacaactggtgggagatcctcacgtcctttatctgcattcaggtcaggattctctaaggggatatttgacattgtgccattaccatcaaagaatgagctgaaagagctgaccgctccgctgttgctaaaactcgtgggtgttttagcttgcgcgttccttattgttccatctgcagatgcagttgatgcacttaaaacttgtgcatgcttattgaagggatgcaggatagaactcgcaaagtgcattgccaaccctgcctgtgcagccaatgtcgcgtgccttcagacctgcaataaccgtccagatgaaaccgagtgccagattaaatgtggggatctgtttgagaacagtgttgttgatgagttcaacgagtgtgctgtgtcgagaaaaaagtgtgttcctagaaaatctgatctcggagaatttcctgccccagacccttctgttcttgtacagaacttcaacatctcggactttaacgggaagtggtacattacaagtggcttgaatccaacctttgatgccttcgactgccagctgcatgagttccacacagaaggtgacaacaagcttgttggaaacatctcttggagaataaagaccctagacagtggattctttactaggtcagccgtacaaaaattcgtgcaagatcctaaccaacctggtgttctctacaatcatgacaacgagtaccttcactatcaagatgactggtatatcctgtcatcaaagatagagaataaacctgaagactatatatttgtatactaccgtgggcgaaacgatgcttgggatggatatggtggtgcagttgtatacacgagaagttctgtattacccaatagcattataccagaactcgaaaaagcagcaaaaagcataggcagagacttcagcacattcattagaacggataacacatgtggtcctgaacctgcgctcgtggagagaattgagaagacagtggaagaaggtgaaaggataatcgtaaaagaggttgaagagatagaagaagaggtagagaaggaagtggagaaggtcggtaggactgagatgaccttgttccagagattggctgaaggatttaatgaactgaagcaagacgaggagaatttcgtgagagagttaagtaaagaagagatggagtttttggatgagatcaaaatggaagcaagtgaggttgaaaaattgtttgggaaagctttgccaatcaggaaggtcaggtagaaacaagaaccaccattgttgtacaaactatattatacatactgtgttcggttcatataaagtaatatttttgtacacagtcatcatcattccataacaattggatacagaaaacacaaggattaaacatcctttgagcgaaac

SEQ ID NO: 4 - protein, 265 aa, Arabidopsis thaliana
MAQTMLLTSGVTAGHFLRNKSPLAQPKVHHLFLSGNSPVALPSRRQSFVPLALFKPKTKAAPKKVEKPKSKVEDGIFGTSGGIGFTKANELFVGRVAMIGFAASLLGEALTGKGILAQLNLETGIPIYEAEPLLLFFILFTLLGAIGALGDRGKFVDDPPTGLEKAVIPPGKNVRSALGLKEQGPLFGFTKANELFVGRLAQLGIAFSLIGEIITGKGALAQLNIETGIPIQDIEPLVLLNVAFFFFAAINPGNGKFITDDGEES

SEQ ID NO: 5 - protein, 667 aa, Arabidopsis thaliana
MGSTPFCYSINPSPSKLDFTRTHVFSPVSKQFYLDLSSFSGKPGGVSGFRSRRALLGVKAATALVEKEEKREAVTEKKKKSRVLVAGGGIGGLVFALAAKKKGFDVLVFEKDLSAIRGEGKYRGPIQIQSNALAALEAIDIEVAEQVMEAGCITGDRINGLVDGISGTWYVKFDTFTPAASRGLPVTRVISRMTLQQILARAVGEDVIRNESNVVDFEDSGDKVTVVLENGQRYEGDLLVGADGIWSKVRNNLFGRSEATYSGYTCYTGIADFIPADIESVGYRVFLGHKQYFVSSDVGGGKMQWYAFHEEPAGGADAPNGMKKRLFEIFDGWCDNVLDLLHATEEEAILRRDIYDRSPGFTWGKGRVTLLGDSIHAMQPNMGQGGCMAIEDSFQLALELDEAWKQSVETTTPVDVVSSLKRYEESRRLRVAIIHAMARMAAIMASTYKAYLGVGLGPLSFLTKFRVPHPGRVGGRFFVDIAMPSMLDWVLGGNSEKLQGRPPSCRLTDKADDRLREWFEDDDALERTIKGEWYLIPHGDDCCVSETLCLTKDEDQPCIVGSEPDQDFPGMRIVIPSSQVSKMHARVIYKDGAFFLMDLRSEHGTYVTDNEGRRYRATPNFPARFRSSDIIEFGSDKKAAFRVKVIRKTPKSTRKNESNNDKLLQTA

SEQ ID NO: 6 - protein, 462 aa, Arabidopsis thaliana
MAVATHCFTSPCHDRIRFFSSDDGIGRLGITRKRINGTFLLKILPPIQSADLRTTGGRSSRPLSAFRSGFSKGIFDIVPLPSKNELKELTAPLLLKLVGVLACAFLIVPSADAVDALKTCACLLKGCRIELAKCIANPACAANVACLQTCNNRPDETECQIKCGDLFENSVVDEFNECAVSRKKCVPRKSDLGEFPAPDPSVLVQNFNISDFNGKWYITSGLNPTFDAFDCQLHEFHTEGDNKLVGNISWRIKTLDSGFFTRSAVQKFVQDPNQPGVLYNHDNEYLHYQDDWYILSSKIENKPEDYIFVYYRGRNDAWDGYGGAVVYTRSSVLPNSIIPELEKAAKSIGRDFSTFIRTDNTCGPEPALVERIEKTVEEGERIIVKEVEEIEEEVEKEVEKVGRTEMTLFQRLAEGFNELKQDEENFVRELSKEEMEFLDEIKMEASEVEKLFGKALPIRKVR

SEQ ID NO: 7 - protein, 46 aa, Arabidopsis thaliana
QLNLETGIPIYEAEPLLLFFILFTLLGAIGALGDRGEAEPLLLFFI

SEQ ID NO: 8 - protein, 49 aa, Arabidopsis thaliana
IGGLVFALAAKRKGFEVLVFEKDLSAVRGEGQYRGPIQIQSNALAALEA

SEQ ID NO: 9 - protein, 56 aa, Arabidopsis thaliana
CAANIACLQTCNNRPDETECQIKCGDLFENNVVDEFNECAVSRKKCVCAVSRKKCV

SEQ ID NO: 10 - protein, 272 aa, Cucumis melo
MAAQTMLLTSGVCVGHGVCLKRELSLRPNNNQFTRLFFNPLPNHSVSLPARGFTPLAVFKSRTKAPPKKVEKPKQKVEDGIFGTSGGIGFTKQNELFVGRVAMIGFAASLLGEAITGKGILAQLNLETGIPIYEAEPLLLFFILFTLLGAIGALGDRGKFIDDPEPATGLERAVIPPGKSFRSALGLKEGGPLFGFTKANELFVGRLAQLGFAFSLIGEIITGKGALAQLNIETGVPINEIEPLVLLNVVFFFIAAVNPGTGKFVTDEEDDE

SEQ ID NO: 11 - protein, 272 aa, Cucumis sativus
MAAQTMLLTSGVCVGHGVCLKRELSLRPNYTQFTRLFFNPLPSHSVSLPPRGFTTLAVFKSRTKAPPKKVEKPKQKVEDGIFGTSGGIGFTKQNELFVGRVAMIGFAASILGEAITGKGILAQLNLETGIPIYEAEPLLLFFILFTLLGAIGALGDRGKFIDDPEPATGLERAVIPPGKSFRSALGLKEGGPLFGFTKANELFVGRLAQLGFAFSLIGEIITGKGALAQLNIETGVPINEIEPLVLLNVVFFFIAAVNPGTGKFVTDEEDDE

SEQ ID NO: 12 - protein, 267 aa, Eutrema salsugineum
MAQTMMLTSGVSANQFLRNKNPLAQPKVHHLFLSGNSPVVIPSRRQSLVPLALFKPKTKAAPKKVEKVKPKVEDGIFGTSGGIGFTKANELFVGRVAMIGFAASLLGEAVTGKGILAQLNLETGIPIYEAEPLLLFFILFTLLGAIGALGDRGKFVDDPPTPTGLEKAVIAPGKNVRSALGLKEQGPLFGFTKANELFVGRLAQLGIAFSLIGEIITGKGALAQLNIETGIPIQDIEPLVLLNVAFFFFAAINPGNGKFITDDGEDM

SEQ ID NO: 13 - protein, 265 aa, Arabidopsis thaliana; identical to SEQ ID NO: 4

SEQ ID NO: 14 - protein, 265 aa, Arabidopsis lyrata
MAQTMLLTSGVSAGQFLRNKSPLAQPKVHHLFLSGNSPVVLPSRRQSFVPLALFKPKTKAAPKKVEKPKKKVEDGIFGTSGGIGFTKANELFVGRVAMIGFAASLLGEALTGKGILAQLNLETGIPIYEAEPLLLFFILFTLLGAIGALGDRGQFVDDPPTGLEKAVIPPGKNVRSALGLKEQGPLFGFTKANELFVGRLAQLGIAFSLIGEIITGKGALAQLNIETGIPIQDIEPLVLLNVAFFFFAAINPGNGKFITDDGEES

SEQ ID NO: 15 - protein, 265 aa, Camelina sativa
MAQTMLLTSGVSAGQFLRNKNPLAQPKVHHLFLSGTSPVALPSRRQSFVPLALFKPKTKAAPKKVVKPKDKVEDGIFGTSGGIGFTKANELFVGRVAMIGFAASLLGEALTGKGILAQLNLETGIPIYEAEPLLLFFILFTLLGAIGALGDRGKFVDDPPTGLEKAVIPPGKGVRSALGLKEQGPLFGFTKANELFVGRLAQLGIAFSLIGEIITGKGALAQLNIETGIPIQDIEPLVLLNVAFFFFAAINPGNGKFITDDGEES

SEQ ID NO: 16 - protein, 265 aa, Capsella rubella
MAQTMLLTSGVSAGQFLRNKNPLAQPKVHQLFLSGTSPVALPSRRQSFVPLALFKPKTKAAPKKVEKVKPKVEDGIFGTSGGIGFTKANELFVGRVAMIGFAASLLGEGITGKGILAQLNLETGIPIYEAEPLLLFFILFTLLGAIGALGDRGKFVDDPPTGLEKAVIPPGKGVRSALGLKEQGPLFGFTKANELFVGRLAQLGIAFSLIGEIITGKGALAQLNIETGIPIQDIEPLVLLNVAFFFFAAINPGNGKFITDDGEES

SEQ ID NO: 17 - protein, 265 aa, Noccaea caerulescens
MAQTMLLTSGVSANQFLRNKNPLAQPKIQHLFLSGNSPVALPSRRPSFVPLALFKPKTKAAPKKVEKAKPKVEDGIFGTSGGIGFTKQNELFVGRVAMIGFAASLLGEALTGKGILAQLNLETGIPIYEAEPLLLFFILFTLLGAIGALGDRGKFVDDPPTGLEKAVIPPGKSVRSALGLKEQGPLFGFTKSNELFVGRLAQLGIAFSLIGEIITGKGALAQLNIETGIPIQDIEPLVLLNVAFFFFAAINPGNGKFITDDGEES

SEQ ID NO: 18 - protein, 265 aa, Brassica napus
MAQTMLLTSGISANHFLRNKNPLAQPKVHHLFLSGNSPVTLPSRIPSLVPLAIFKPKTKAAPKKVEKVKPKVEDGIFGTSGGIGFTKQNELFVGRVAMIGFAASLLGEALTGKGILAQLNLETGIPIYEAEPLLLFFILFTLLGAIGALGDRGKFVDDPPTGLEKAVIPPGKGVRSALGLKEQGPLFGFTKANELFVGRLAQLGIAFSLIGEIITGKGALAQLNIETGIPIQDIEPLVLLNVAFFFAAAINPGNGKFITDDGEES

SEQ ID NO: 19 - protein, 265 aa, Raphanus sativus
MAQTMLLTSGISANHFLRNKNPLAQPKVHHLFLSGNSPVTLPSRRPSLVPLAIFKPKTKAAPKKVEKVKPKVEDGIFGTSGGIGFTKQNELFVGRVAMIGFAASLLGEALTGKGILAQLNLETGIPIYEAEPLLLFFILFTLLGAIGALGDRGKFVDDPPTGLEKAVIPPGKGVRSALGLKEQGPLFGFTKANELFVGRLAQLGIAFSLIGEIITGKGALAQLNIETGIPIQDIEPLVLLNVAFFFFAAINPGNGKFITDDGEES

SEQ ID NO: 20 - protein, 265 aa, Brassica rapa
MAQTMLLTSGISANHFLRNKNPLAQPKVHHLFLSGNSPVTLPSRRPSLVPLAIFKPKTKAAPKKVEKVKPKVEDGIFGTSGGIGFTKQNELFVGRVAMIGFAASLLGEALTGKGILAQLNLETGIPIYEAEPLLLFFILFTLLGAIGALGDRGKFVDDPPTGLEKAVIPPGKGVRSALGLKEQGPLFGFTKANELFVGRLAQLGIAFSLIGEIITGKGALAQLNIETGIPIQDIEPLVLLNVAFFFAAAINPGNGKFITDDGEES

SEQ ID NO: 21 - protein, 265 aa, Raphanus sativus
MAQTMLLTSGVSANTFLRNKNPLAQPKVHHLFLSGNSHVILPSRRPSLVPLAIFKPKTKAAPKKVEKVKPKVEDGIFGTSGGIGFTKQNELFVGRVAMIGFAASLLGEALTGKGILAQLNLETGIPIYEAEPLLLFFILFTLLGAIGALGDRGKFVDDPPTGLEKAVIPPGKGVRSALGLKEQGPLFGFTKANELFVGRLAQLGIAFSLIGEIITGKGALAQLNIETGIPIQDIEPLVLLNVAFFFFAAINPGNGKFITDDGEES

SEQ ID NO: 22 - protein, 265 aa, Brassica napus
MAQTMLLTSGVSANQFLRNKNPLAQPKVHHFFLSGNSHVVLPSRRPSLVPLAIFKPKTKAAPKKVEKVKPKVEDGIFGTSGGIGFTKQNELFVGRVAMIGFAASLLGEALTGKGILAQLNLETGIPIYEAEPLLLFFILFTLLGAIGALGDRGKFVDDPPTGLEKAVIPPGKGVRSALGLKEQGPLFGFTKANELFVGRLAQLGIAFSLIGEIITGKGALAQLNIETGIPIQDIEPLVLLNVAFFFFAAINPGNGKFITDDGEES

SEQ ID NO: 23 - protein, 265 aa, Brassica rapa
MAQTMLLTSGVSANQFLRNKNPLAQPKVHHFFLSGNSHVVLPSRRPSLVPLAIFKPKTKAAPKKVEKVKPKVEDGIFGTSGGIGFTKQNELFVGRVAMIGFAASLLGEALTGKGILAQLNLETGIPIYEAEPLLLFFILFTLLGAIGALGDRGKFVDDPPTGLEKAVIPPGKGVRSALGLKEQGPLFGFTKANELFVGRLAQLGIAFSLIGEIITGKGALAQLNIETGIPIQDIEPLVLLNVAFFFFAAINPGNGKFITDDGEER

SEQ ID NO: 24 - protein, 274 aa, Phoenix dactylifera
MVHAVFTSGLGAHLPDSKREPLLQSQLRRLRPTPFSHLLLSQPSHKQLPSPSYSSYTPVLALFKSKTKAPPKKVEKAKPKVEDGIFGTSGGIGFTKQNELFVGRVAMIGFAASLLGEAITGKGILAQLNLETGIPIYEAEPLLLFFILFTLLGAIGALGDRGRFVDDPPTGLDKAVIPPGKGIRSALGLKEGGPLFGFTKSNELFVGRLAQLGIAFSIIGEIVTGKGALAQLNIETGVPINEIEPLVLFNVIFFFIAALNPGNGKFVTDVDEEE

SEQ ID NO: 25 - protein, 270 aa, Anthurium amnicola
MAQSMLMSSLGSRLVETKGEPLLQFQIRRLRPTPATHLLLPPPTRRHPLPPSYAPTLAAFKSKTKAAPKKVEKGNFKVEDGIFGTSGGIGFTKQNELFVGRVAMIGFAASLLGEAITGKGILAQLNLETGIPIYEAEPLLLFFILFTLLGAIGALGDRGRFVDDPPTGLDKAVVPPGKGFRSSLGLKEGGPLFGFTKSNELFVGRLAQLGIAFSIIGEIITGKGALAQLNIETGVPISDIEPLVLLNVVFFFLAALNPGTGQFVTDDGED

SEQ ID NO: 26 - protein, 269 aa, Trifolium subterraneum
MAQTMLLMSSVSSTYSVELKKDPLLQLQCQRLRSRISDVSFNPLSSNSKSLSSRTFTTLALFKSKTKAPAKVVKPKPKVEDGIFGTSGGFGFTKQNELFVGRVAMIGFAASILGEALTGKGILAQLNLETGIPIYEAEPLLLFFIIFTLLGAIGALGDRGKFVDDEPTTGGVIPPGKGFRAALGLREGGPLFGFTKSNELFVGRLAQLGFVFSLIGEIITGKGALAQLNVETGVPITEIEPLVLFNVIFFFIAALNPGTGTFVTDEEED

SEQ ID NO: 27 - protein, 270 aa, Pisum sativum
MAQTMLLMSSVSSTYSVPLNKDPLLQLQCQRLKPRFSDISFSPLSSNSKSFSSRTFKTLALFKSKTKAPAKVVPKQKPKVEDGVFGTSGGFGFTKQNELFVGRVAMIGFAASILGEGITGKGILSQLNLETGIPIYEAEPLLLFFIIFTLLGAIGALGDRGKFVDDEPTTGGVIPPGKGFRQALGLSEGGPLFGFTKSNELFVGRLAQLGFAFSLIGEIITGKGALAQLNIETGVPINEIEPLVLFNVAFFFIAALNPGTGKFVTDEEED

SEQ ID NO: 28 - protein, 271 aa, Beta vulgaris
MAQAMLLMPSVSTTNTIDLKRNALLKIQIQKIKPKSSSSHLFFSPLSSSSSSSSTFKTLALFKPKTKAPVKKVEKPKLKVEDGLFGTSGGIGFTKENELFVGRVAMIGFAASLLGEGLTGKGILAQLNLETGIPIYEAEPLLLFFILFTLLGAIGALGDRGRFVDDPPTGLEKAVIPPGKNVRSALGLREGGPLFGFTKSNELFVGRLAQLGFAFSLIGEIITGKGALAQLNIETGVPVNEIEPLVLLNVLFFFIAAINPGTGKFITDEEE

SEQ ID NO: 29 - protein, 274 aa, Cephalotus follicularis
MAQTMLLMCGISTSHVVDLRRDPLFHVQIQKLRPKSFSHLFFNPLSNNGFSLAQKFNTLALFKSKTKAAPKKVATTAKPKVEDGLFGTSGGIGFTKQNELFVGRVAMIGFAASLLGEAVTGKGILSQLNLETGIPIYEAEPLLLFFILFTLLGAIGALGDRGRFVDDEPTGLERAVIPPGKGIRGALGLREGGPLFGFTKSNELFVGRLAQLGIAFSLIGEIITGKGALAQLNIETGIPINEIEPLVLFNVIFFFFAALNPGTGKFVTDEEAED

SEQ ID NO: 30 - protein, 665 aa, Tarenaya hassleriana
MGSTLFCSPVNPSLSKLDFSRTHLLSPADKHFFLDLPSFMGKVRGKSSVMSRRRVVGVKATAAVEEERRETAAEKEKLRVLVAGGGIGGLVFALAAKRKGFDVAVFEKDLSAIRGEGQYRGPIQIQSNALAALEAIDMGVAEEVMEAGCITGDRINGLVDGVSGSWYVKFDTFTPAAERGLPVTRVISRMTLQQILARAVGEDVIQNESNVVSFSESEDKVTVVLENGECYQGDLLVGADGIWSKVRSQLFGHEEATYSGYTCYTGIADFVPADIESVGYRVFLGHKQYFVSSDVGGGKMQWYAFHEEPAGGRDAPDGRKKRLLEIFQGWCDNVIDLLHATEEDAILRRDIYDRTPSFTWGKGRVTLLGDSIHAMQPNMGQGGCMAIEDSYQLAWELEHAWRRSVETDKPIDIVSSLRSYEEARKLRVAIIHGMARMAAIMASTYKGYLGVGLGPLSFLTMLRIPHPGTVGGRFFIDVAMPLMLNWVLGGNSSKLEGRLPCCRLSDKADDQLQRWFQDNDALERTVIGDWYLIPYGNDSIVSETVRLDKDEDQPCIIGSEPDEDFPGMRIEIPSSQVSKVHARIIYKDGAFFVMDLRSEYGTYITDNEGRRYRVTPNFPARFRPSDIIELGSDKKAAFRVKVIRKTPKMTRRDDRESSSKLLQAA

SEQ ID NO: 31 - protein, 663 aa, Arabis alpina
MGSTPFCYTINPSPSKLDFTKTHLAKQFYLDLSSFTGKSGAGLSGIKNRRGVVGVKASATALVEEEKRETVTEKKKKSRVLVAGGGIGGLVFALAAKKKGFDVLVFEKDLSAIRGEGQYRGPIQIQSNALAALEAIDIAVAEEVMEAGCITGDRINGLVDGVSGTWYVKFDTFTPAASRGLPVTRVISRMTLQQILARAVGEEVIRNESNVVDFEDSGDKVTVVLENGQRYEGDLLVGADGIWSKVRNNLFGRSEATYSGYTCYTGIADFIPADIESVGYRVFLGHKQYFVSSDVGGGKMQWYAFYEEPAGGVDAPNGMKKRLFDIFEGWCDNVLDLLHATEEEAILRRDIYDRSPSFTWGKGRVTLLGDSIHAMQPNMGQGGCMAIEDSYQLASELEDAWKQSVDTNRPVDVVSSLKRYEESRRLRVAIIHGMARMAAIMASTYKAYLGVGLGPLSFLTKFRVPHPGRVGGRFFIDIAMPLMLNWVLGGNSEKLEGRAPSCRLTDRADDRLREWFDDNEALERTISGEWYLIPQGDDCCVSETLCLTKDEDQPCIIGSEPDKDFPGMHIVIPSSQVSKMHARIIYKDGAFFVMDLRSEHGTYVVDNEGGRYRATPNFPARFRPSDILEFGSDKKAAFKVKVIRKTPKSTSKNESNGKLLQAA

SEQ ID NO: 32 - protein, 665 aa, Camelina sativa
MGSTPFCYSINPSPSKLDFTRTHVFSPVSKQFYLDLSSFTGKSAGGGGGFRSRRALVGVKAATALVEEKRESGTEKKKKSRVLVAGGGIGGLVFALAAKKKGFDVLVFEKDLSAIRGEGQYRGPIQIQSNALAALEAIDTDVAEQVMEAGCITGDRINGLVDGISGTWYVKFDTFTPAASRGLPVTRVISRMTLQQILARAVGEEVIRNESNVVDFEDSGDKVTVVLENGERYEGDLLVGADGIWSKVRNNLFGRSEASYSGYTCYTGIADFIPADIESVGYRVFLGNKQYFVSSDVGGGKMQWYAFHEEPAGGADAPNGMKKRLFEIFDGWCDNVLDLLHATEEDAILRRDIYDRNPSFTWGKGRVTLLGDSIHAMQPNMGQGGCMAIEDSFQLALELDEAWKQSVETKTPVDVVSSLKRYEESRRLRVALIHGMARMAAIMASTYKAYLGVGLGPLSFLTKFRVPHPGRVGGRFFIDIAMPMMLNWVLGGNSEKLEGRSPSCRLTDKADDRLREWFEDDDALERTIKGEWYLIPHGDDCCISETLCLTKDEDQPCIIGSEPDQDLPGKHIVIPSSQVSKMHARVIYKDGAFFLMDLRSEHGTYVTDNEGRRYRATPNSPARFRTSDIIEFGSDKKAAFRVKVIRTTPKSTRKNESNDKLLQAA

SEQ ID NO: 33 - protein, 668 aa, Camelina sativa
MGSTPFCYSINPTPSKLDFTRTHVFSPVSKQFYLDLSSFTGKSGVGAGGFRSLRALVGVKAATALVEEEQKRESVTDKTKKKSRVLVAGGGIGGLVFALAAKKKGFDVLVFEKDLSAIRGEGQYRGPIQIQSNALAALEAIDTDVAEQVMVAGCITGDRINGLVDGISGTWYVKFDTFTPAASRGLPVTRVISRMTLQQILARAVGEELIRNESNVVDFEDSGDKVTVVLENGERYEGDLLVGADGIWSKVRNNLFGRSEASYSGYTCYTGIADFIPADIESVGYRVFLGNKQYFVSSDVGGGKMQWYAFHEEPAGGADAPNGMKKRLFEIFDGWCDNVLDLLHATEEDAILRRDIYDRNPSFTWGKGRVTLLGDSIHAMQPNMGQGGCMAIEDSFQLALELDEAWKQSVKTKTPVDVVSSLKRYEESRRLRVALIHGMARMAAIMASTYKAYLGVGLGPLSFLTKFRVPHPGRVGGRFFIDIAMPMMLNWVLGGNSEKLEGRSPSCRLTDKADDRLREWFEDDDALERTIKGEWYLIPHGDECCISETLCLTKDEDQPCIIGSKPDQDLPGKHIVIPSSQVSKMHARVIYKDGAFFLMDLRSEHGTYVTDNEGRRYRATPNSPARFRTSDIIEFGSDKKAAFRVKVIRTTPKSTRKNESNDKLLQAA

SEQ ID NO: 34 - protein, 669 aa, Capsella rubella
MGSTPFCYSINPSPSKLDFTRTHVFSPVAKQFYLDLSSFTGKSGVGGGLSGFRSRRTLVGVKAATALVEEEQKPGEVTERKKKSRVLVAGGGIGGLVFALAAKKKGFDVLVFEKDLSAIRGEGQYRGPIQIQSNALAALEAIDNDVAEQVMEAGCITGDRINGLVDGVSGTWYVKFDTFTPAASRGLPVTRVISRMTLQQILARAVGEEVIRNESNVVDFEDSGDKVTVVLENGQRYEGDLLVGADGIWSKVRNNLFGRSEAEYSGYTCYTGIADFIPADIESVGYRVFLGHKQYFVSSDVGGGKMQWYAFHEEPAGGTDAPNGMKKRLFEIFDGWCDNVLDLLHATEEDAILRRDIYDRSPSFTWGKGRVTLLGDSIHAMQPNMGQGGCMAIEDSFQLALELEEAWKQSVETNTSVDVVSSLKKYEESRRLRVAIIHGMARMAAIMASTYKAYLGVGLGPLSFLTKFRVPHPGRVGGRFFIDIAMPLMLNWVLGGNSEKLEGRPPSCRLTDKADDRLREWFENDDALERTINGEWYLIPHGDECCVSETLCLTKDEDQPCIVGSEPDQDLPGKHIVIPSSQVSKMHARVIYKDGAFFLMDLGSEHGTFVTDNEGRRYRATPNFPGRFRSSDIIEFGSDKKAAFRVKVIRKTPKATRKNESNDKLLQAA

SEQ ID NO: 35 - protein, 667 aa, Arabidopsis thaliana; identical to SEQ ID NO: 5

SEQ ID NO: 36 - protein, 667 aa, Arabidopsis lyrata
MGSTLFCYSINPSPSKLDFTRTHVVSPVAKQFYLDLSSFSGKSGGGLSGFRSRKTLVGVKAATALVEKEEKREAVTEKKKKSRVLVAGGGIGGLVFALAAKKKGFDVVVFEKDLSAIRGEGQYRGPIQIQSNALAALEAIDTDVAEQVMEAGCITGDRINGLVDGVSGSWYVKFDTFTPAASRGLPVTRVISRMTLQQILARAVGEDVIRNESNVVDFEDSGDKVTVVLENGQRYEGDLLVGADGIWSKVRNNLFGRSEATYSGYTCYTGIADFVPADIESVGYRVFLGHKQYFVSSDVGGGKMQWYAFHEEPAGGVDAPNGMKKRLFEIFDGWCDNVLDLLHATEEDAILRRDIYDRSPSFTWGKGRVTLLGDSIHAMQPNMGQGGCMAIEDSFQLALELEEAWKQSVGTNTPVDVVSSLKRYEESRRLRVAIIHGMARMAAIMASTYKAYLGVGLGPLSFLTKFRVPHPGRVGGRFFVDIAMPLMLDWVLGGNSEKLEGRPPSCRLTDKADDRLREWFEDDDALERTIKGEWYLIPHGEDCCVSETLCLTNDEDQPCIVGSEPDQDFPGMRIVIPSSQVSKMHARVIYKDGVFFLMDLRSEHGTYVTDNEGRRYRATPNFPARFRSSDIIEFGSDKKAAFRVKVIRKTPKSTRKNESNDKLLQTA

SEQ ID NO: 37 - protein, 662 aa, Raphanus sativus
MGSSTLFCYSINPSPSKLDFTKTHVFSPVAKQFYLDFPSFAAGKLRLRKRRALVGAKAETLLEEKRETVTEKKKKPRVLVAGGGIGGLVFALAAKKKGFDVLVFEKDLSAIRGEGQYRGPIQIQSNALAALEAIDIGVAEEVMEAGCITGDRINGLVDGVSGTWYVKFDTFTPAASRGLPVTRVISRMTLQQILARAVGEEIIRNESNVVDFQDSGDKVTVVLENGERYDGDLLVGADGIWSKVRNNLFGRSEATYSGYTCYTGIADFVPADIESVGYRVFLGHKQYFVSSDVGGGKMQWYAFHEEAAGGVDAPNGMKKRLFDIFEGWCDNVLDLLQATEEEAILRRDIYDKSPSFTWGKGRVTLLGDSIHAMQPNMGQGGCMAIEDSFQLGLELEAAWKQSVETNTPVDVVSSLRRYEESRRLRVAIIHGMARMAAIMASTYKAYLGVGLGPLSFLTKFRVPHPGRVGGRFFIDIAMPLMLNWVLGGNSEKLEGRPPSCRLTDKADDRLREWFEDDEALERTINGEWYLIPHGNECSVSETLRLTKDEEQPCIVGSEPDQDFPGTHIVIPSPQVSKMHARVIYKDGAFFLMDLRSEHGTYLTDNEGGKYRVTPNFPTRFRSSDIIEFGSDKKAAFRVKVIRTTPKLTRRDEKSDGKLLQAA

SEQ ID NO: 38 - protein, 687 aa, Brassica napus
MKCTSHIKLPLRASRIEMGSSTPFCYSINPSPSKLDFTRTHAFSPVAKQFYLDLPSFAGKSGGGLSGLRKRRTLIGVKAAAATLVAEEEKRETVTESKKKPRVLVAGGGIGGLVFALAAKKKGFDVLVFEKDLSAIRGEGQYRGPIQIQSNALAALEAIDIGVAEEVMEAGCITGDRINGLVDGVSGTWYVKFDTFTPAASRGLPVTRVISRMTLQQILARAVGEEIIRNESNVVDFEDSGDKVTVVLENGQRYDGDLLVGADGIWSKVRNNLFGRSEATYSGYTCYTGIADFVPADIESVGYRVFLGHKQYFVSSDVGGGKMQWYAFHEEAAGGVDAPNGMKKRLFDIFEGWCDNVLDLLQATEEEAILRRDIYDRSPSFTWGKGRVTLLGDSIHAMQPNMGQGGCMAIEDSFQLGLELEQAWKQSVETNTPVDVVSSLRRYEESRRLRVAIIHGMARMAAIMASTYKAYLGVGLGPLSFLTKFRVPHPGRVGGRFFIDIAMPLMLNWVLGGNSEKLEGRPPSCRLTDKADDRLREWFEDDEALERTINGEWYLIPHGNECSVSETLRLTKDEDQPCIVGSEPDQDFPGMHIVIPSPQVSKMHARVIYKDGAFFVMDLRSEHGTYLTDNEGGKYRVTPNFPARFRPSDIIEFGSDKKAAFRVKVIRTTPKLTRRDEKSDGKLLQAA

SEQ ID NO: 39 - protein, 668 aa, Brassica rapa
MGCSTPFCYSINPSPSKLDFTKTHAFSPVAKQFYLDLPSFAGKSGGGLSGLRKRRALVGVKAATLLAEEEKRETVTESKKKPRVLVAGGGIGGLVFALAAKKKGFDVLVFEKDLSAIRGEGQYRGPIQIQSNALAALEAIDIGVAEEVMEAGCITGDRINGLVDGVSGTWYVKFDTFTPAASRGLPVTRVISRMTLQQILARAVGEEIIRNESNVVDFEDSGDKVTVVLENGQRYDGDLLVGADGIWSKVRNNLFGRSEATYSGYTCYTGIADFVPADIESVGYRVFLGHKQYFVSSDVGGGKMQWYAFHEEAAGGVDAPNGMKKRLFDIFEGWCDNVLDLLQATEEEAILRRDIYDRSPSFTWGKGRVTLLGDSIHAMQPNMGQGGCMAIEDSFQLGLELEQAWKQSVETNTPVDVVSSLRRYEESRRLRVAIIHGMARMAAIMASTYKAYLGVGLGPLSFLTKFRVPHPGRVGGRFFIDIAMPLMLNWVLGGNSEKLEGRPPSCRLTDKADDRLREWFEDDEALERTINGEWYLIPHGNECSVSETLRLTKDEEQPCIVGSEPDQDFPGTHIVIPSPQVSKMHARVIYKDGAFFVMDLRSEHGTYLTDNEGGKYRVTPNFPARFRPSDIIEFGSDKKAAFRVKVIRTTPKLTRRDEKSDGKLLQAA

SEQ ID NO: 40 - protein, 668 aa, Brassica rapa
MGCSTPFCYSINPSPSKLDFTKTHAFSPVAKQFYLDLPSFAGKSGGGLSGLRKRRALVGVKAATLLAEEEKRETVTESKKKPRVLVAGGGIGGLVFALAAKKKGFDVLVFEKDLSAIRGEGQYRGPIQIQSNALAALEAIDIGVAEEVMEAGCITGDRINGLVDGVSGTWYVKFDTFTPAASRGLPVTRVISRMTLQQILARAVGEEIIRNESNVVDFEDSGDKVTVVLENGQRYDGDLLVGADGIWSKVRNNLFGRSEATYSGYTCYTGIADFVPADIESVGYRVFLGHKQYFVSSDVGGGKMQWYAFHEEAAGGVDAPNGMKKRLFDIFEGWCDNVLDLLQATEEEAILRRDIYDRSPSFTWGKGRVTLLGDSIHAMQPNMGQGGCMAIEDSFQLGLELEQAWKQSVETNTPVDVVSSLRRYEESRRLRVAIIHGMARMAAIMASTYKAYLGVGLGPLSFLTKFRVPHPGRVGGRFFIDIAMPLMLNWVLGSNSEKLEGRPPSCRLTDKADDRLREWFEDDEALERTINGEWYLIPHGNECSVSETLRLTKDEEQPCIVGSEPDQDFPGTHIVIPSPQVSKMHARVIYKDGAFFVMDLRSEHGTYLTDNEGGKYRVTPNFPARFRPSDIIEFGSDKKAAFRVKVIRTTPKLTRRDEKSDGKLLQAA

SEQ ID NO: 41 - protein, 667 aa, Noccaea caerulescens
MGSTPFCYSTNPSPSKLDFTRTHAFSPLAKQFYLDLSSLAGKSGGGLSGFRSPRTLVGVKAAAATALVEEEKREVVAEKKKSRVLVAGGGIGGLVFALAAKKKGFDVLVFEKDLSAIRGEGQYRGPIQIQSNALAALEAIDTDVAEEVMEAGCITGDRINGLVDGVSGTWYVKFDTFTPAASRGLPVTRVISRMTLQQILARAVGEEIIRNESNVVDFEDSGDKVTVVLENGERYEGDLLVGADGIWSKVRNNLFGRSEATYSGYTCYTGIADFVPADIESVGYRVFLGHKQYFVSSDVGGGKMQWYAFHEEPAGGVDPPNGMKKRLFDIFEGWCDNVLDLLHATEEDAILRRDIYDRTPSFTWGKGRVTLLGDSIHAMQPNMGQGGCMAIEDSYQLAMELEGAWKQSVETNTPVDVVSSLKKYEESRRLRVAIIHGMARMAAIMASTYKAYLGVGLGPLSFLTKFRVPHPGRVGGRFFIDIAMPLMLNWVLGGNSEKLEGRSPSCRLTDKADDRLREWFEDNDALERTINGEWYLIPHGDDSSVKETISLTKDEDQPCIIGSEPDQDLPGMHIVIPSSQVSKMHARVTYKDGAFFLMDLGSEHGTYVVDNEGRRYRASPNYPARFRSSDIIEFGSDKKAAFRVKVIRTTPKSTSKNESNGKLLQAA

SEQ ID NO: 42 - protein, 666 aa, Eutrema salsugineum
MGSTPFCYSINPSPSKLDFTRTHVFSPVAKQFYLDLSSCAGKSGGGLSGFRSRRALVGVRAATALVEEEKREIAKEKKKPRVLVAGGGIGGLVFALAAKKKGFDVLVFEKDLSAIRGEGQYRGPIQIQSNALAALEAIDIDVAEEVMEAGCITGDRINGLVDGVSGTWYVKFDTFTPAASRGLPVTRVISRMTLQQILARAVGEEVIRNESNVVDFEDSGDKVTVVLENGERYEGDLLVGADGIWSKVRNNLFGRSEATYSGYTCYTGIADFVPADIESVGYRVFLGHKQYFVSSDVGGGKMQWYAFHEEPAGGVDAPNGMKKRLFDIFEGWCDNVLDLLHATEEEAILRRDIYDRTPSFNWGKGRVTLLGDSIHAMQPNMGQGGCMAIEDSYQLALELEEAWERSVETNAPVDVVSSLRRYEESRRLRVAIIHGMARMAAIMASTYKAYLGVGLGPLSFLTKFRVPHPGRVGGRFFIDIAMPLMLNWVLGGNSEKLEGRPPSCRLTDKADDRLREWFEDDDALERTINGEWYLIPYGNECSVSETLCLTKDEDQPCIIGSEPDQDFPGMHIVIPAPQVSKMHARVTYKDGAFFLMDLRSEHGTYVTDNEGRRYRVTPNFPARFRSSDIIEFGSDKKAAFRVKVIRTTPKSTSKNKESNGKLLQAV

SEQ ID NO: 43 - protein, 666 aa, Eutrema halophilum
  VARIANT 492: Xaa = Any Amino Acid
MGSTPFCYSINPSPSKLDFTRTHVFSPVAKQFYLDLSSCAGKSGGGLSGFRSRRALVGVRAATALVEEEKREIAKEKKKPRVLVAGGGIGGLVFALAAKKKGFDVLVFEKDLSAIRGEGQYRGPIQIQSNALAALEAIDIDVAEEVMEAGCITGDRINGLVDGVSGTWYVKFDTFTPAASRGLPVTRVISRMTLQQILARAVGEEVIRNESNVVDFEDSGDKVTVVLENGERYEGDLLVGADGIWSKVRNNLFGRSEATYSGYTCYTGIADFVPADIESVGYRVFLGHKQYFVSSDVGGGKMQWYAFHEEPAGGVDAPNGMKKRLFDIFEGWCDNVLDLLHATEEEAILRRDIYDRTPSFNWGKGRVTLLGDSIHAMQPNMGQGGCMAIEDSYQLALELEEAWERSVETNAPVDVVSSLRRYEESRRLRVAIIHGMARMAAIMASTYKAYLGVGLGPLSFLTKFRVPHPGRVGGRFFIDIAMPLMLNWVLGXNSEKLEGRPPSCRLTDKADDRLREWFEDDDALERTINGEWYLIPYGNECSVSETLCLTKDEDQPCIIGSEPDQDFPGMHIVIPAPQVSKMHARVTYKDGAFFLMDLRSEHGTYVTDNEGRRYRVTPNFPARFRSSDIIEFGSDKKAAFRVKVIRTTPKSTSKNKESNGKLLQAV

SEQ ID NO: 44 - protein, 665 aa, Cucumis sativus
MALTRFHNPFNLSSSSLSRTCFPVPAFREYLVEISPCQRIGCNFGGKSACGRRKKLTQVKAAVTEAPPAEGAAGEISRSLPTKNVRILVAGGGIGGLVFALAAKRKGFDVVVFEKDISAIRGEGQYRGPIQIQSNALAALEAIDLDVAEEVMRVGCITGDRINGLVDGVSGNWYIKFDTFTPAAERGLPVTRVISRMSLQQILARAVGDDVIINDSNVVDFEDSGEKVKVTLENGQQHEGDLLVGADGIWSKVRKNLFGHSEAVYSGYTCYTGIADFIPADIETVGYRVFLGHKQYFVSSDVGAGKMQWYAFHKEPPGGADAPNGKKERLFKIFEGWCDNVTDLIQATDEDSVLRRDIYDRTPIFTWGKGRVTLLGDSVHAMQPNMGQGGCMAIEDGYQLALELDKAWNESVASGSPIDIVSSLKSYESSRRIRVAVIHGMARMAALMASTYKAYLGVGLGPLSFLTQFRIPHPGTFGGRFFIDLAMPLMLNWVLGGNSSKLEGRPPACRLSDKANDQLRKWFEDDDALERAINGDWFLLPQGGEASVSQPICLRKDENQPCLIGSVEKEVDSGLSVAIPLPQVSEKHARIYYKDGAFFLTDLRSEHGTWLSDHEGRRYRAPPNFPVRFHQSDLIEFGSDKKARFRVKVIRSSVENDREKVEMNS

SEQ ID NO: 45 - protein, 658 aa, Vitis vinifera
MASAVFYSSVQPSIFSRTHIPIPISKDSFEEFGHSINYKHYFRSNPCGQKKRVAQVKATLAEATPAPPAPSLPSKKVRILVAGGGIGGLVLALAAKKKGFDVVVFEKDMSAIRGEGQYRGPIQIQSNALAALEAVDMEVAEEVMRAGCITGDRINGLVDGVSGDWYVKFDTFTPAAERGLPVTRVISRMTLQQILARAVGEDIIMNGSNVVDFEDDGNKVTVILENGQRYEGDLLIGADGIWSKVRKSLFGPKEATYSGYTCYTGIADFVPADIDSVGYRVFLGHKQYFVSSDVGAGKMQWYAFYNEPAGGVDGPEGKKERLLKIFGGWCDNVIDLILATDEEAILRRDIYDRTPTFTWGRGRVTLLGDSVHAMQPNMGQGGCMAIEDSYQLAMELDKAWEQSIKSGTPIDVVSCLKSYEKARRIRVAVIHGMARMAAIMASTYKAYLGVGLGPLSFLTKLRIPHPGRVGGRFFIDIAMPLMLSWVLGGNSSKLEGRPPSCRLSDKANDQLRRWFEDDDALERAIGGEWFLLPSGESGLQPICLSKDENKPCIIGSVSHTDFPGISTVIPSPKVSKMHARISCKDGAFFLTDLQSEHGTWITDNVGRRQRVSPNFPTRFHPSEVIDFGSEKASFRVKVVRTPPDNAAKNEESKLFQAV

SEQ ID NO: 46 - protein, 664 aa, Corchorus olitorius
MATTLFQNPSTFFTGTQFPVSIPKYVPTESSACLHCNYHFRGKASKQKKRFLQVKATVAGTQSDSKSDEKNKVDANQQEKKKARILVAGGGIGGLVFALAAKNKGFDVVVFEKDLSAIRGEGQYRGPIQIQSNALAALEAIDMEVAEKVMEAGCITGDRINGLVDGVSGSWYIKFDTFTPAAERGLPVTRVISRMTLQQILARAVGEDIIFNESNVVDFEDDGNKVSVVLENGKRFEGDLLVGADGIWSKVRKNLFGPKDAVYSGYTCYTGIADFVPADIDSVGYRVFLGHKQYFVSSDVGGGKMQWYAFHKEPAGGVDTQGKKERLLKIFEGWCDNVIDLLLATDEEAILRRDIYDRTPSLTWGKGRVTLLGDSIHAMQPNLGQGGCMAIEDGYQLALELDKAWKQSVESGTPIDVVSSLRSYESARRLRVAIIHGMARMAAIMASTYKAYLGVGLGPLSFLTKYRIPHPGRVGGRFFIDIAMPLMLSWVLGGNSSKLEGRSLTCRLSDKASDQLREWFEDNDALERAISGEWFLFPAGDGVSSQPICLSRDENNPFMIGSEKKEDFPGTSVVIPSSQVSKTHAQITYKDGAFFVTDLQSEHGTYIINQEGKKSRVTPNVPTRIRPSDVIEFGSDKKAAFRVKAIKSAPKIAEKEGSGVLQAA

SEQ ID NO: 47 - protein, 661 aa, Populus euphratica
MASSTLFGNTLTAVSSRTHFPTPIFNNSLELLSSTHSNYNFKTKTSTSAKKLKVEAVVTETPAVSKSEGKQSEQRKLKVLVAGGGIGGLVFALAAKNKGFDVMVFEKDLSAVRGEGQYRGPIQIQSNALAALEAIDLDVAEEVMRAGCITGDRINGLVDGISGTWYVKFDTFTPAAERGLPVTRVISRMTLQQILARSVGDDTILNDSNVVSFQDDGDKVTVVLENGQQYEGDLLVGADGIWSKVRKNLFGPKEAVYSGYTCYTGIADFVPVDIETVGYRVFLGHKQYFVSSDVGAGKMQWYAFHKESPGGMDAPHGKKDRLLKIFEGWCDNVIDLLLTTDEDSILRRDIYDREPIITWGKGRVTLLGDSVHAMQPNMGQGGCMAIEDSYQLASELERAWKQSIESGTPVDVLSSLRSYENARRLRVAIIHGMARMAAIMASTYKAYLGVGLGPLSFLTNFRIPHPGRVGGRFFIDIAMPVMLDWVLGGNSSKLEGRSLSCRLSDKASDQLRRWFVDDDALERSLNGEWFLLPCGNDAVASQPIGLSRDENKPCVVGSVSQEDFPGMSIVIPAPQVSKTHARITCKDGAFYLIDLRSEHGTFITDIEGRRYRAPPNFPTRFHPSDMIEFGSDKKVIFRVKVMRSPPKISEKKDEGQVLQSV

SEQ ID NO: 48 - protein, 665 aa, Ricinus communis
MASSAFFCNSINPSTSVFSRTHFSFPIFSTSTVEFSSFAQYNFHFKTKKSDHQNKRFTQVKAVVTESPTVAESNGKLSEQKKLRILVAGGGIGGLVFALAAKRKGFEVLVFEKDLSAIRGEGQYRGPIQVQSNALAALEAIDLEVAEEVMRAGCITGDRINGLVDGVSGTWYCKFDTFTPAAERGLPVTRVISRMTLQQILACAVGEDVIMNASNVINFQDNEDKVTVTLENGQQFEGDLLVGADGIWSKVRKNLFGPKEATYSGYTCYTGIADFVPVDIESVGYRVFLGHKQYFVSSDVGAGKMQWYAFHNEPPGGVDSPNGKKERLLKIFEGWCDNVIDLLHATDEDAILRRDIYDREPVFTWGKGRVTLLGDSIHAMQPNMGQGGCMAIEDSYQLALELDKAWKQSIESGTPVDVVSSLKSYERTRRLRVAIIHGMARMAAIMASTYKAYLGVGLGPLSFLTKYRIPHPGRVGGRFFIDIAMPVMLNWVLGGNSSKLEGRPLSCRLSDKASDQLQTWFEDDNALERALNGEWFLLPFGDDAVQEPICLSRDENIPCMVGSESQEDFPGKSIVISSPQVSKMHARISYKDGGFYVIDLQSEHGTFITDNDGRRSRVPPNFPTLFHPSEAIEFGSAGKAKFRVKVMKSPAKIKEKGGNEILQSV

SEQ ID NO: 49 - protein, 665 aa, Jatropha curcas
MASSTLFCNLINPSISVFSRTHLPFPIVSSSSMELSSSAHCNFHFRSKKSEQNKKLTQVKAVVTESTSVAQSDEKQPEQRKPRILVAGGGIGGLVFALAAKRKGFEVLVFEKDLSAVRGEGQYRGPIQIQSNALAALEAIDLEVAEEVMEAGCITGDRINGLVDGVSGTWYVKFDTFTPAAERGLPVTRVISRMTLQQILALAVGEDVIRNESNVVSFQDDGDKVTVTLENGQHFEGDLLVGADGIWSKVRKNLFGPKDATYSDYTCYTGIADFVPADIESVGYRVFLGHKQYFVSSDVGAGKMQWYAFHKEPPGGVDRPNGKKERLLKIFEGWCDNVIDLLLATDEDAILRRDIYDRTPTLTWGRGRVTLLGDSVHAMQPNMGQGGCMAIEDGYQLALEIEKAWKQSIESGTPIDIVSSLKSYERARRLRVAIIHGMARMAAIMASTYKAYLGVGLGPLSFLTKYRIPHPGRVGGRFFIDIAMPVMLSWVLGGNSSKLEGRSQCCRLSDKASDQLRTWFEDDDALERALNAEWFLLPLGNKVVVSEPICLSRNENTPCVVGKVSHKDFPGMSIVIPSPQVSEMHARISYKDGAFYVIDLQSEHGTYISDADGRRYRVPQNSPTRFHPSDVIEFGSDEKAKFRVKVMKSPSRIKEKEGSEILQSV

SEQ ID NO: 50 - protein, 480 aa, Eucalyptus grandis
MASMAAGSICLFRDESIGAASIAVTILANRSSHMAKLLCYRGKARATMWMGIKTTRRLAMKCSLESHCRSESSCSGFPLPRKEEVTSSRGSRSGVPKVTESAREIFHLVREWSQRRVIQLAALAACTFLIIPSADAVDALKTCACLLKECRIELAKCVANPSCAANVACLQTCNNRPDETECQIKCGDLFENSVVDEFNECAVSRKKCVPRKSDVGEFPVPDPAVLVKSFNMADFTGKWFISSGLNPTFDTFDCQLHEFHTESNKLMGNLTWRIRTPDSGFFTRTAVQRFVQDPEQPGILYNHDNEYLHYQDDWYILSSKTENKPDDYVFVYYRGRNDAWDGYGGAVVYTRSAVLPDSIVPELERAAKSVGRDFKDFIRTDNTCGPEPPLVERIEKTVEEGEKTIVREVEQIEDEVQKVGKTEMTLFQRLTEGFRELRQDEENFLRRLSQEEMEVLNELKMEATEVEKLFGRALPIRKLR

SEQ ID NO: 51 - protein, 458 aa, Tarenaya hassleriana
MAVAVQSFSSPCYRDTQFISGNRSNRKLLRKRMVDSDTIVLVKICSGARGKIHCSLKARFSSPSSGYKSGLSKGRPPFEALTLWNKLKEQSRQSLLKLVGILACTFLIVPSVDAVDALKTCACLLKECRIELAKCISNPSCAANVACLQTCNNRPDETECQIKCGDLFENSVVDEFNECAVSRKKCVPRKSDLGEFPAPDPAVLVKRFNIGDFSGKWYISSGLNPTFDTFDCQLHEFHTESDKLVGNLSWRIRTPDGGFFTRSTVQKFVQDPNQPGILYNHDNEYLHYQDDWYILSSKVENGPDDYVFVYYRGRNDAWDGYGGAVVYTRSAVLPNNIVPELERAAKSVGRDFSKFIRTDNTCGPEPPLVERIEKTVEEGERTIIREVEQIEGEVAKVGETEMTLLQRLVEGFKELKQDEENFLQGLNKEEMELLSELKMEASEVEKLFGKALPIRKLR

SEQ ID NO: 52 - protein, 461 aa, Camelina sativa
MAVATHCFTSPCHDRIRFFSSDDGIGRLGISRKRINGTFLVKILPPIQNVDLRTNGRSSRPLSAFRSGISKGVFDILSLPSKDELKELSTPLLLKLVGVFACAFLIVPSAEAVDALKTCACLLKGCRIELAKCISNPACAANIACLQTCNNRPDETECQIKCGDIFENKVVDEFNECAVTRKKCVPKKSDLGEFPAPDPSVLVQNFNIGDFSGKWYITSGLNPTFDAFDCQLHEFHTEGENKLVGNISWRIKTLDSGFFTRSAVQTFVQDPNQPGVLYNHDNEYLHYQDDWYILSSKIENKPEDYIFVYYRGRNDAWDGYGGAVVYTRSSVLPNSIVPELEKAAKSIGRDFSTFIRTDNTCGPEPPLVERLEKTVEEGERIIVKDFEEIEEEVEKEVEKVGKTEMTLFQRLAEGFNELRKDEENFVRELSKEEMEFLDEIKMEANEVEKLFGKALPIRKVR

SEQ ID NO: 53 - protein, 461 aa, Capsella rubella
MAVATHCFTSPCHDRIRFFSSDDGIARLGISRKRINGTFLVKILSPIQSADLRTSGRSSRPLSAFRSGFSKRVFDIVSLPSKNELKELSTPLLLKLVGVLACAFLIVPSAEAVDALKTCACLLEGCRIELAKCIANPACAANVACLQTCNNRPDETECQIKCGDLFENSVVDEFNECAVSRKKCVPRKSDLGEFPAPDPSVLVQNFNIGDFNGKWYITSGLNPTFDAFDCQLHEFHTEGDNKLVGNISWRIKTLDSGFFTRSAVQTFVQDPNQPGVLYNHDNAYLHYQDDWYILSSKIENKPEDYIFVYYRGRNDAWDGYGGAVVYTRSSVLPNSIVPELEKAAKSIGRDFSTFIKTDNTCGPEPPLVERLEKTVEEGERIIVKEVEEIEEEVEKEVEKVGKTEMTLFQRLAEGFNELKQDEENFVRELSKEEMEFLDEIKMEASEVEKLFGKALPIRKVR

SEQ ID NO: 54 - protein, 462 aa, Arabidopsis thaliana; identical to SEQ ID NO: 6

SEQ ID NO: 55 - protein, 455 aa, Arabidopsis lyrata
MAVATHCFTSPCHGRIRFFSSDDGRLGITRKRINGTFLLKILPPIQNAGGRSSRPISAFRSGFSKGIFDIVALPSKNELKELTTPLLLKLVGVLACAFLIVPSADAVDALKTCACLLKGCRIELAKCIANPACAANVACLQTCNNRPDETECQIKCGDLFENSVVDEFNECAVSRKKCVPRKSDLGEFPAPDPSVLVQNFNISDFNGKWYITSGLNPTFDAFDCQVHEFHTEGDNKLVGNISWRIKTLDSGFFTRSAVQKFVQDPNQPGVLYNHDNEYLHYQDDWYILSSKIENKPDDYIFVYYRGRNDAWDGYGGAVVYTRSSVLPNSIIPELEKAAKSIGRDFSTFIRTDNTCGPEPPLVERIEKTVEEGERIIVKEVEEIEEEVEKEVEKVGKTEMTLFQRLAEGFNELKQDEENFVREFSKEEMEFLDEIKMEASEIEKLFGKALPIRKVR

SEQ ID NO: 56 - protein, 457 aa, Brassica napus
MSVSTHCFTSPCHDRTRFFSGDDGNKLLRKRIKGTFLVKILPSSQNAYLRITAKSSRPLSGFRSGISKGVFDIVALTSKNALKELTTPLMLKLVGVVACAFLIVPSADAVDALKTCACLLKGCRIELAKCIANPSCAANVACLQTCNNRPDETECQIKCGDLFENSVVDEFNECAVSRKKCVPRKSDLGEFPAPDPSVLVKNFNINDFDGKWYITSGLNPTFDAFDCQLHEFHTEDGKLVGNISWRIKTPDSGFFTRSTVQKFVQDPNQPAVFYNHDNEYLHYQDDWYILSSKIENKPEDYIFVYYRGRNDAWDGYGGAVVYTRSASLPNTIVPELEKAAKSIGREFSTFIKTDNTCGPEPPLVERLEKTVEEGEKIIVKEVEEIEEEVEKEVEKVGKTEMTLFQRLAEGFEELKQDEENFLRGLSKEEMELLDELKMEANEVEKLFGKALPIRKFR

SEQ ID NO: 57 - protein, 491 aa, Brassica rapa
MSYPKGISSHPYISLFLFSLYLPPLLPAELSVSSMSVSTHCFTSPCHDRTRFFSGDDGNKLLRKRIKGTFLVKILPSSQNAYLRVTAKSSRPLSGFRSGISKGVFDIVALTSKNALKELSTPLMLKLVGVVACAFLIVPSADAVDALKTCACLLKGCRIELAKCIANPSCAANVACLQTCNNRPDETECQIKCGDLFENSVVDEFNECAVSRKKCVPRKSDLGEFPAPDPSVLVKNFNVKDFDGKWYITSGLNPTFDAFDCQLHEFHTEDGKLVGNISWRIKTPDSGFFTRSTVQKFVQDPNQPAVFYNHDNEYLHYQDDWYILSSKIENKPEDYIFVYYRGRNDAWDGYGGAVVYTRSASLPNTIVPELEKAAKSIGREFSTFIKTDNTCGPEPPLVERLEKTVEEGEKIIVKEVEEIEEEVEKEVEKVGKTEMTLFQRLAEGFEELKQDEENFLRGLSKEEMELLDELKMEANEVEKLFGKALPIRKFR

SEQ ID NO: 58 - protein, 493 aa, Noccaea caerulescens
LSLSLSLSLSLSLLPAELSIFGIASGRLATESMSVATHCFTSPTCHDRIRFFSRITSDDGRLVRKRINGTFLLKILPPSQNAHLRTTLRSSRPLSAGFRSGISKGVIDIVALTSRNALKELSTPLLLKLVGVLACAFLIVPSADAVDALKTCACLLKECRIELAKCIANPSCAANVACLQTCNNRPDETECQIKCGDLFANSVVDEFNECAVSRKKCVPRKSDLGEFPVPDPSALVKNFNIQDFNGKWYITSGLNPTFDIFDCQLHEFHVQGNKLVGNISWRIKTPDTGFFTRSAVQTFKQDPNQPAVLYNHDNEYLHYQDDWYILSSKIENKPEDYIFVYYRGRNDAWDGYGGAVVYTRSNVLPNSIVPELEKAAKSIGRDFNTFVRTDNTCGPEPPLVERLEKTVEEGEKMIEKEVEEIEEEVEKEVEKVGKTEMTLFQRLAEGFNELKQDEENFLRGLSEEEMALLDELKMEAGEVEKLFGKALPIRKFR

SEQ ID NO: 59 - protein, 459 aa, Eutrema salsugineum
MAVATYCFTSPCHDRIRFFSGVTSFDGRLLRKRINGTFLVKILPPSQNADLRTTSRSSRPLSGFRSGTSKGVFDIVALTSRNALKELSTPMVLKLVGVLACAFLIVPSADAVDALKTCACLLKGCRIELAKCIANPSCAANVACLQTCNNRPDETECQIKCGDLFENKVVDEFNECAVSRKKCVPQKSDLGEFPVPDPSVLVKNFNISDFNGKWYITSGLNPTFDTFDCQRHEFHADGDKLVGNISWRIKTLDSGFFTRSAVQKFVQDPNQPAILYNHDNEYLHYQDDWYILSSKVENKPDDYIFVYYRGRNDAWDGYGGAVVYTRSAVLPNSIVPELEKAAKSIGRDFSTFVRTDNTCGPEPPLVERFEKTVEEGEKIIVKEVEEIEEEVEKEVEKVGKTEMTLFQRLAEGFNELKQDEENFLRGLSEEEMELLNELKMEASEVEKLFGKSLPIRKVR

SEQ ID NO: 60 - protein, 481 aa, Prunus humilis
MALAGRSIFLSHNDSIGNTCIRLGITSDEGFQKRRMVGFHVVVKFPSNRRKSRYSQFIRSKRNFCVLGSKCSSLLSSKTEEAFSKCSTRTSEPEMKRVISFLLEEASSCIKEWSQLHFMKVAGLLACTFMIMPSANAADALKTCACLLKECRVELAKCIGNPSCAANIACLQTCNNRPDETECQIKCGDLFENSVVDEFNECAVSRKKCVPKKSDVGEFPIPDPAVLVKSFDIEKFNGKWFITSGLNPTFDAFDCQLHEFHTESSKLVGNLSWRIRTPDGGFFTRSAVQKFVQDPNQPGILYNHDNDYLHYQDDWYILSSKMENKPDDYIFVYYRGRNDAWDGYGGAVIYTRSSVLPASIVPDLEKAAASVGRDFSKFIRTDNTCGPEPPLVERLEKTLEEGERNIIEEVKQIEGEVEKVEQTELTLLQKLAEGFNELKQDEENFLRGLSKEEMDILSELKMEAGEVEKLFGQTLPLRKLR

SEQ ID NO: 61 - protein, 481 aa, Pyrus x bretschneideri
MAFAGRSVFLSHKESIGNACIRLGLKSDERLQKGRMVGFHVVVKFSSQRRKSRYCQFISAKRNFSGLGSKRSSLLSSRTEEAFSERSTKTSEPEMGRAIDLMIEEVLSVIKEWSQLHFMKVAGLLLCTFMVMPSANAVDALKTCACLLKECRVELAKCIGNPSCAANIACLQTCNNRPDETECQIKCGDLFENKVVDEFNECAVSRKKCVPMKSDVGEFPIPDPAALVKSFDMSKFNGKWFITSGLNPTFDVFDCQLHEFHTESSKLVGNLSWRIKTPDGGFFTRSAVQKFVQDPNQPGILYNHDNEYLHYQDDWYILSSKIENTPEDYIFVYYRGRNDAWDGYGGAVVYTRSSVLPESIVPELERAAKSVGRDFSKFIRTDNTCGPEPPLVERLEKTIEEGERTIIEEVKQIEGEVEKVEQTELTLFQKLLEGFNVLKQDEENFLRGLSKEEMDLLSELKMEAGEVGKLFGKTLPLRKLR

SEQ ID NO: 62 - protein, 471 aa, Bixa orellana
MALAPHSTHFSELTGRRFLSRKVVHLHGMVLLRIQSSDRKSRYSKSINPYRNHIVSKLRCSDQLSEGTHNISSTCSSNTRRKHEAKEGFEFVVPNLPNILRKWSQLQIMKVAGVLACALLVIPSASAVDALKTCTCLLKECRIELAKCIANPSCAANVACLQTCNNRPDETECQIKCGDLFENSVVDVFNECAVSRKKCVPQKSDVGEFAVPDPSVLVKNFNIADFSGKWYISSGLNPSFDTFDCQLHEFHTESNKLVGNLSWRIRTPDGGFFTRSTLQKFVQDPKQPGILYNHDNEYLHYQDDWYILSSKIENKQDDYVFVYYRGRNDAWDGYGGAVVYTRSAVLPESIVPELERAAKCVGRDFNKFIKTDNTCGPEPPLVERLEKKVEEGEETIIREVEQLEGQVEKVGKTEMTLFQKLAEGFKELQKDEENFLEELSKEEMDVLSELKMEAREVEKLFGGALPLRKLR

SEQ ID NO: 63 - protein, 487 aa, Theobroma cacao
MAQAARSLCFSHDKSVQVPCRTSGLTSNERFHRRQIAHFHGIMLVKIQSSGRKARYSQLNKSNPNYSASDLRCSNQLSRRKDRNFSSCSCNRRRPKAEEAFAFLVPTISNVLKEWSQSKIVKVVGLLACAYLVIPSASAVDALKTCTCLLKECRIELAKCIANPSCAANIACLQTCNDRPDETECQIKCGDLFENSVVDEFNECAVSRKKCVPQKSDIGEFPVPSPAVLVKNFNIADFSGKWFISSGLNPTFDTFDCQLHEFHTEAGKLVGNLSWRIGTPDGGFFTRSTLQRFVQDPNYPGILYNHDNEYLHYQDDWYIISSKIENKQDDYIFVYYQGRNDAWDGYGGAVVYTRSAVLPESIVPELEKAAKNVGRDFNKFIRTDNTCGPEPPLVERLEKKVEEGEQTLIREVKEIEGEVEKEVKRVEKTEMTLFQKLAEGFKELQQDEENFLRGLSKEEMGLLNELKMEASEVEKLFGEALPLRKLR

SEQ ID NO: 64 - protein, 479 aa, Gossypium arboreum
MAEAARLICFSHGKSVKVPCRTSGFTRKERFHRRLVAHFHGMMLLKLQSSCRNSRYSQLIKPNMNYSASKLRCSHQLSRRKERKFSSSSSNERTPKIPTISNLLEQWSQSQTVKLVGLLACAYLVIPSAAAVDALKTCTCLLKECRIELAKCIANPSCAANVACLQTCNDRPDETECQIKCGDLFENSVVDEFNECAVSRKKCVPQKSDIGEFPVPDPAVLVENFNIADFTGKWFISSGLNPTFDTFDCQLHEFHIEGGKLVGNLSWRIRTPDGGFFTRSATQRFVQDPNHPGILYNHDNEYLHYQDDWYIISSKIENKPDDYVFVYYRGRNDAWDGYGGAVVYTRSAVLPETIVPELKRAAQNVGRNFNKFIRTDNSCGPEPPLVERLEKKVEEGEQTLIREVEQIEGEVEKGVEKVEKTEQTLFQRLAEGFKELQQDEENFLRGLSKEEMELLNDLKMEASEVEKLFGEALPIRKLR

SEQ ID NO: 65 - protein, 487 aa, Gossypium hirsutum
MAEAARLICFSHGKSVKVPCRTSGFTRKERFHRRLVAHFHGMMLLKLQSSCRNSRYSQLIKPNMNYSASKLRCSHQFSRRKERKFSSSSSNERTPKAEEVFSFQIPTISNLLEQWSQSQTVKLVGLLACAYLVIPSAAAVDALKTCTCLLKECRIELAKCIANPSCAANVACLQTCNDRPDETECQIKCGDLFENSVVDEFNECAVSRKKCVPQKSDIGEFPVPDPAVLVENFNIADFTGKWFISSGLNPTFDTFDCQLHEFHIEGGKLVGNLSWRIRTPDGGFFTRSATQRFLQDPNHPGILYNHDNEYLHYQDDWYIISSKIENKPDDYVFVYYRGRNDAWDGYGGAVVYTRSAVLPETIVPELKRAAQNVGRNFNKFIRTDNSCGPEPPLVERLEKKVEEGEQTLIREVEQIEGEVEKGVEKVEKTEQTLFQRLAEGFKELQQDEENFLRGLSKEEMELLNDLKMEASEVEKLFGEALPIRKLR

SEQ ID NO: 66 - protein, 489 aa, Populus trichocarpa
MALAANPFCLSQEQYIISSSSVAKSGLASDGRFHRRQRLHFHGAVLSQFWPNSRKLRYIQSIRSHRHHYGGVIRCSNQLSDWTKKFSSLCSSSSRSMPKAIERLNFVVLSVTNALKERNNLECLKLAGILLCALLVIPSADAVDALKTCTCLLKECRLELAKCIANPSCAANVACLQTCNNRPDETECQASSIKCGDLFENSVVDEFNECAVSRKKCVPRKSDVGEFPVPDPAVLVENFNMADFSGKWFITSGLNPTFDTFDCQLHEFHTESNKLVGNLSWRIKTPDTGFFTRSAVQRFVQDPVHPGILYNHDNEYLHYQDDWYILSSKIENKQDDYVFVYYQGRNDAWDGYGGAVVYTRSAVLPESIVPELEKAAKSVGRDFSKFIRTDNTCGPEPPLVERLEKTVEEGEKTIIKEVEEIEQKVEKAGKTELSLFQRLTEGFKEIQKDEENFLRELSKEETDLLNDLRMEAGEVEKLFGRALPIRKLR

SEQ ID NO: 67 - protein, 483 aa, Manihot esculenta
MAISANSVCLSHEESICSSYFRPGIASYERIHGRRGLNYQSIVVLNFWPNSRKSRYVQLMRTHKNYHGIKLRCSHGFSGWTKKFSSFCRTGANVTKAKEVLNFLMFSVSNNLKEKSHLQFLKVASILACVLLFIPSADAVDALKTCTCLLKECRLELAKCIANPACAANIACLQTCNNRPDETECQIKCGDLFENTVVDEFNECAVSRKKCVPKKSDVGEFPVPDPAVLVKSFNIADFNGKWYITRGLNPTFDTFDCQLHEFHVESNKLVGNISWRIRTPDSGFFTRSTVQRFVQDPMQPGILYNHDNEYLHYQDDWYILSSKVENKSDDYIFVYYRGRNDAWDGYGGAVVYTRSSVLPESIAPELERAAKSVGRDFSKFIRTDNTCGPEPPLVERLEKTVEEGEKSIIREVQEIEGEVEKVGKTEMTLFQRLAEGFKELQQDEEILLRKLSKEEMELFNDLKMEASEVEKLFGGALPLRKLR

SEQ ID NO: 68 - protein, 481 aa, Jatropha curcas
MALAANSIYLSHEESISSSYIKSGIERFHGRKGLHFRSIVVLKILPNSRKSRRHVQLIRSYRNYCGLVLRCSHQFSGWTNKFPSFSSTAASINKAKEVLNFLMLSVSNNLKEKGQLQFLKVAGILACALLVIPSADAVDALKTCACLLKECRLELAKCIANPACAANIACLQTCNNRPDETECQIKCGDLFENNVVDEFNECAVSRKKCVPKKSDVGEFPVPDPAVLVKSFNIADFSGKWFITSGLNPTFDTFDCQLHDFHRESNRLVGNLSWRIRTPDGGFFTRSTVQKFVQDPLQPGILYNHDNEYLHYQDDWYILSSKLENSENDYIFVYYRGRNDAWDGYGGAVVYTRSAVLPESIIPELETAAKKVGRDFNKFIITDNTCGPEPPLAERIEKTVEEGEKTIIREVEEIEGNVEKVGKTEMALFQRLAEGFKELQQDEEFFVRELSKEEMDILNDLKMEAGEVEKLFGEALPLRKLR